European Patent Specification EP 3 286 570 B1, published July 1, 2026. Title: A method for predicting the risk of incidence of chronic kidney disease. Applicant: sphingotec GmbH. The sequence listing filed with the application follows.

SEQUENCE LISTING (12 sequences)

SEQ ID NO: 1 - protein, 243 aa, Homo sapiens
ECSQDCATCSYRLVRPADINFLACVMECEGKLPSLKIWETCKELLQLSKPELPQDGTSTLRENSKPEESHLLAKRYGGFMKRYGGFMKKMDELYPMEPEEEANGSEILAKRYGGFMKKDAEEDDSLANSSDLLKELLETGDNRERSHHQDGSDNEEEVSKRYGGFMRGLKRSPQLEDEAKELQKRYGGFMRRVGRPEWWMDYQKRYGGFLKRFAEALPSDEEGESYSKEVPEMEKRYGGFMRF

SEQ ID NO: 2 - protein, 73 aa, Homo sapiens
ECSQDCATCSYRLVRPADINFLACVMECEGKLPSLKIWETCKELLQLSKPELPQDGTSTLRENSKPEESHLLA

SEQ ID NO: 3 - protein, 5 aa, Homo sapiens
YGGFM

SEQ ID NO: 4 - protein, 5 aa, Homo sapiens
YGGFL

SEQ ID NO: 5 - protein, 20 aa, Homo sapiens
MDELYPMEPEEEANGSEILA

SEQ ID NO: 6 - protein, 41 aa, Homo sapiens
DAEEDDSLANSSDLLKELLETGDNRERSHHQDGSDNEEEVS

SEQ ID NO: 7 - protein, 8 aa, Homo sapiens
YGGFMRGL

SEQ ID NO: 8 - protein, 12 aa, Homo sapiens
SPQLEDEAKELQ

SEQ ID NO: 9 - protein, 11 aa, Homo sapiens
VGRPEWWMDYQ

SEQ ID NO: 10 - protein, 22 aa, Homo sapiens
FAEALPSDEEGESYSKEVPEME

SEQ ID NO: 11 - protein, 28 aa, Homo sapiens
FAEALPSDEEGESYSKEVPEMEKRYGGF

SEQ ID NO: 12 - protein, 7 aa, Homo sapiens
YGGFMRF